European Patent Application EP 4 353 833 A1, published April 17, 2024. Title: Origami-fingerprinting based diagnostics. Applicant: University of Fribourg. The sequence listing filed with the application follows.

SEQUENCE LISTING (300 sequences)

SEQ ID NO: 1 - DNA, 8063 bp, synthetic construct
  source 1..8063: mol_type = other DNA
tgatagacggtttttcgccctttgacgttggagtccacgttctttaatagtggactcttgttccaaactggaacaacactcaaccctatctcgggctattcttttgatttataagggattttgccgatttcggaaccaccatcaaacaggattttcgcctgctggggcaaaccagcgtggaccgcttgctgcaactctctcagggccaggcggtgaagggcaatcagctgttgcccgtctcactggtgaaaagaaaaaccaccctggcgcccaatacgcaaaccgcctctccccgcgcgttggccgattcattaatgcagctggcacgacaggtttcccgactggaaagcgggcagtgagcgcaacgcaattaatgtgagttagctcactcattaggcaccccaggctttacactttatgcttccggctcgtatgttgtgtggaattgtgagcggataacaatttcacacaggaaacagctatgaccatgattacgaattcgagctcggtacccggggatcctcaactgtgaggaggctcacggacgcgaagaacaggcacgcgtgctggcagaaacccccggtatgaccgtgaaaacggcccgccgcattctggccgcagcaccacagagtgcacaggcgcgcagtgacactgcgctggatcgtctgatgcagggggcaccggcaccgctggctgcaggtaacccggcatctgatgccgttaacgatttgctgaacacaccagtgtaagggatgtttatgacgagcaaagaaacctttacccattaccagccgcagggcaacagtgacccggctcataccgcaaccgcgcccggcggattgagtgcgaaagcgcctgcaatgaccccgctgatgctggacacctccagccgtaagctggttgcgtgggatggcaccaccgacggtgctgccgttggcattcttgcggttgctgctgaccagaccagcaccacgctgacgttctacaagtccggcacgttccgttatgaggatgtgctctggccggaggctgccagcgacgagacgaaaaaacggaccgcgtttgccggaacggcaatcagcatcgtttaactttacccttcatcactaaaggccgcctgtgcggctttttttacgggatttttttatgtcgatgtacacaaccgcccaactgctggcggcaaatgagcagaaatttaagtttgatccgctgtttctgcgtctctttttccgtgagagctatcccttcaccacggagaaagtctatctctcacaaattccgggactggtaaacatggcgctgtacgtttcgccgattgtttccggtgaggttatccgttcccgtggcggctccacctctgaaagcttggcactggccgtcgttttacaacgtcgtgactgggaaaaccctggcgttacccaacttaatcgccttgcagcacatccccctttcgccagctggcgtaatagcgaagaggcccgcaccgatcgcccttcccaacagttgcgcagcctgaatggcgaatggcgctttgcctggtttccggcaccagaagcggtgccggaaagctggctggagtgcgatcttcctgaggccgatactgtcgtcgtcccctcaaactggcagatgcacggttacgatgcgcccatctacaccaacgtgacctatcccattacggtcaatccgccgtttgttcccacggagaatccgacgggttgttactcgctcacatttaatgttgatgaaagctggctacaggaaggccagacgcgaattatttttgatggcgttcctattggttaaaaaatgagctgatttaacaaaaatttaatgcgaattttaacaaaatattaacgtttacaatttaaatatttgcttatacaatcttcctgtttttggggcttttctgattatcaaccggggtacatatgattgacatgctagttttacgattaccgttcatcgattctcttgtttgctccagactctcaggcaatgacctgatagcctttgtagatctctcaaaaatagctaccctctccggcattaatttatcagctagaacggttgaatatcatattgatggtgatttgactgtctccggcctttctcacccttttgaatctttacctacacattactcaggcattgcatttaaaatatatggggttctaaaaatttttatccttgcgttgaaataaaggcttctcccgcaaaagtattacagggtcataatgtttttggtacaaccgatttagctttatgctctgaggctttattgcttaattttgctaattctttgccttgcctgtatgatttattggatgttaatgctactactattagtagaattgatgccaccttttcagctcgcgccccaaatgaaaatatagctaaacaggttattgaccatttgcgaaatgtatctaatggtcaaactaaatctactcgttcgcagaattgggaatcaactgttatatggaatgaaacttccagacaccgtactttagttgcatatttaaaacatgttgagctacagcattatattcagcaattaagctctaagccatccgcaaaaatgacctcttatcaaaaggagcaattaaaggtactctctaatcctgacctgttggagtttgcttccggtctggttcgctttgaagctcgaattaaaacgcgatatttgaagtctttcgggcttcctcttaatctttttgatgcaatccgctttgcttctgactataatagtcagggtaaagacctgatttttgatttatggtcattctcgttttctgaactgtttaaagcatttgagggggattcaatgaatatttatgacgattccgcagtattggacgctatccagtctaaacattttactattaccccctctggcaaaacttcttttgcaaaagcctctcgctattttggtttttatcgtcgtctggtaaacgagggttatgatagtgttgctcttactatgcctcgtaattccttttggcgttatgtatctgcattagttgaatgtggtattcctaaatctcaactgatgaatctttctacctgtaataatgttgttccgttagttcgttttattaacgtagatttttcttcccaacgtcctgactggtataatgagccagttcttaaaatcgcataaggtaattcacaatgattaaagttgaaattaaaccatctcaagcccaatttactactcgttctggtgtttctcgtcagggcaagccttattcactgaatgagcagctttgttacgttgatttgggtaatgaatatccggttcttgtcaagattactcttgatgaaggtcagccagcctatgcgcctggtctgtacaccgttcatctgtcctctttcaaagttggtcagttcggttcccttatgattgaccgtctgcgcctcgttccggctaagtaacatggagcaggtcgcggatttcgacacaatttatcaggcgatgatacaaatctccgttgtactttgtttcgcgcttggtataatcgctgggggtcaaagatgagtgttttagtgtattcttttgcctctttcgttttaggttggtgccttcgtagtggcattacgtattttacccgtttaatggaaacttcctcatgaaaaagtctttagtcctcaaagcctctgtagccgttgctaccctcgttccgatgctgtctttcgctgctgagggtgacgatcccgcaaaagcggcctttaactccctgcaagcctcagcgaccgaatatatcggttatgcgtgggcgatggttgttgtcattgtcggcgcaactatcggtatcaagctgtttaagaaattcacctcgaaagcaagctgataaaccgatacaattaaaggctccttttggagccttttttttggagattttcaacgtgaaaaaattattattcgcaattcctttagttgttcctttctattctcactccgctgaaactgttgaaagttgtttagcaaaatcccatacagaaaattcatttactaacgtctggaaagacgacaaaactttagatcgttacgctaactatgagggctgtctgtggaatgctacaggcgttgtagtttgtactggtgacgaaactcagtgttacggtacatgggttcctattgggcttgctatccctgaaaatgagggtggtggctctgagggtggcggttctgagggtggcggttctgagggtggcggtactaaacctcctgagtacggtgatacacctattccgggctatacttatatcaaccctctcgacggcacttatccgcctggtactgagcaaaaccccgctaatcctaatccttctcttgaggagtctcagcctcttaatactttcatgtttcagaataataggttccgaaataggcagggggcattaactgtttatacgggcactgttactcaaggcactgaccccgttaaaacttattaccagtacactcctgtatcatcaaaagccatgtatgacgcttactggaacggtaaattcagagactgcgctttccattctggctttaatgaggatttatttgtttgtgaatatcaaggccaatcgtctgacctgcctcaacctcctgtcaatgctggcggcggctctggtggtggttctggtggcggctctgagggtggtggctctgagggtggcggttctgagggtggcggctctgagggaggcggttccggtggtggctctggttccggtgattttgattatgaaaagatggcaaacgctaataagggggctatgaccgaaaatgccgatgaaaacgcgctacagtctgacgctaaaggcaaacttgattctgtcgctactgattacggtgctgctatcgatggtttcattggtgacgtttccggccttgctaatggtaatggtgctactggtgattttgctggctctaattcccaaatggctcaagtcggtgacggtgataattcacctttaatgaataatttccgtcaatatttaccttccctccctcaatcggttgaatgtcgcccttttgtctttggcgctggtaaaccatatgaattttctattgattgtgacaaaataaacttattccgtggtgtctttgcgtttcttttatatgttgccacctttatgtatgtattttctacgtttgctaacatactgcgtaataaggagtcttaatcatgccagttcttttgggtattccgttattattgcgtttcctcggtttccttctggtaactttgttcggctatctgcttacttttcttaaaaagggcttcggtaagatagctattgctatttcattgtttcttgctcttattattgggcttaactcaattcttgtgggttatctctctgatattagcgctcaattaccctctgactttgttcagggtgttcagttaattctcccgtctaatgcgcttccctgtttttatgttattctctctgtaaaggctgctattttcatttttgacgttaaacaaaaaatcgtttcttatttggattgggataaataatatggctgtttattttgtaactggcaaattaggctctggaaagacgctcgttagcgttggtaagattcaggataaaattgtagctgggtgcaaaatagcaactaatcttgatttaaggcttcaaaacctcccgcaagtcgggaggttcgctaaaacgcctcgcgttcttagaataccggataagccttctatatctgatttgcttgctattgggcgcggtaatgattcctacgatgaaaataaaaacggcttgcttgttctcgatgagtgcggtacttggtttaatacccgttcttggaatgataaggaaagacagccgattattgattggtttctacatgctcgtaaattaggatgggatattatttttcttgttcaggacttatctattgttgataaacaggcgcgttctgcattagctgaacatgttgtttattgtcgtcgtctggacagaattactttaccttttgtcggtactttatattctcttattactggctcgaaaatgcctctgcctaaattacatgttggcgttgttaaatatggcgattctcaattaagccctactgttgagcgttggctttatactggtaagaatttgtataacgcatatgatactaaacaggctttttctagtaattatgattccggtgtttattcttatttaacgccttatttatcacacggtcggtatttcaaaccattaaatttaggtcagaagatgaaattaactaaaatatatttgaaaaagttttctcgcgttctttgtcttgcgattggatttgcatcagcatttacatatagttatataacccaacctaagccggaggttaaaaaggtagtctctcagacctatgattttgataaattcactattgactcttctcagcgtcttaatctaagctatcgctatgttttcaaggattctaagggaaaattaattaatagcgacgatttacagaagcaaggttattcactcacatatattgatttatgtactgtttccattaaaaaaggtaattcaaatgaaattgttaaatgtaattaattttgttttcttgatgtttgtttcatcatcttcttttgctcaggtaattgaaatgaataattcgcctctgcgcgattttgtaacttggtattcaaagcaatcaggcgaatccgttattgtttctcccgatgtaaaaggtactgttactgtatattcatctgacgttaaacctgaaaatctacgcaatttctttatttctgttttacgtgcaaataattttgatatggtaggttctaacccttccattattcagaagtataatccaaacaatcaggattatattgatgaattgccatcatctgataatcaggaatatgatgataattccgcrccttcrggtggtttctttgttccgcaaaatgataatgttactcaaacttttaaaattaataacgttcgggcaaaggatttaatacgagttgtcgaattgtttgtaaagtctaatacttctaaatcctcaaatgtattatctattgacggctctaatctattagttgttagtgctcctaaagatattttagataaccttcctcaattcctttcaactgttgatttgccaactgaccagatattgattgagggtttgatatttgaggttcagcaaggtgatgctttagatttttcatttgctgctggctctcagcgtggcactgttgcaggcggtgttaatactgaccgcctcacctctgttttatcttctgctggtggttcgttcggtatttttaatggcgatgttttagggctatcagttcgcgcattaaagactaatagccattcaaaaatattgtctgtgccacgtattcttacgctttcaggtcagaagggttctatctctgttggccagaatgtcccttttattactggtcgtgtgactggtgaatctgccaatgtaaataatccatttcagacgattgagcgtcaaaatgtaggtatttccatgagcgtttttcctgttgcaatggctggcggtaatattgttctggatattaccagcaaggccgatagtttgagttcttctactcaggcaagtgatgttattactaatcaaagaagtattgctacaacggttaatttgcgtgatggacagactcttttactcggtggcctcactgattataaaaacacttctcaggattctggcgtaccgttcctgtctaaaatccctttaatcggcctcctgtttagctcccgctctgattctaacgaggaaagcacgttatacgtgctcgtcaaagcaaccatagtacgcgccctgtagcggcgcattaagcgcggcgggtgtggtggttacgcgcagcgtgaccgctacacttgccagcgccctagcgcccgctcctttcgctttcttcccttcctttctcgccacgttcgccggctttccccgtcaagctctaaatcgggggctccctttagggttccgatttagtgctttacggcacctcgaccccaaaaaacttgatttgggtgatggttcacgtagtgggccatcgccc

SEQ ID NO: 2 - DNA, 32 bp, synthetic construct
  source 1..32: mol_type = other DNA
gtctatcatcggaaccgaaaggaagtgctttc

SEQ ID NO: 3 - DNA, 32 bp, synthetic construct
  source 1..32: mol_type = other DNA
cgtggactccaacgtccgctagggtactatgg

SEQ ID NO: 4 - DNA, 24 bp, synthetic construct
  source 1..24: mol_type = other DNA
gaacaagatgcgcgtaccgccgcg

SEQ ID NO: 5 - DNA, 32 bp, synthetic construct
  source 1..32: mol_type = other DNA
aagaatagcccgagatggcggtttcctgtcgt

SEQ ID NO: 6 - DNA, 31 bp, synthetic construct
  source 1..31: mol_type = other DNA
tccgaaatcggcaaattcttttcttgcgctc

SEQ ID NO: 7 - DNA, 32 bp, synthetic construct
  source 1..32: mol_type = other DNA
cccagcaggcgaaaatattgccctctaatgag

SEQ ID NO: 8 - DNA, 32 bp, synthetic construct
  source 1..32: mol_type = other DNA
tggccctgagagagttgtccacgctggtttgc

SEQ ID NO: 9 - DNA, 24 bp, synthetic construct
  source 1..24: mol_type = other DNA
gccagctggggtaaagttctgcca

SEQ ID NO: 10 - DNA, 32 bp, synthetic construct
  source 1..32: mol_type = other DNA
cataaagtggtgccggatcagacgatccagcg

SEQ ID NO: 11 - DNA, 32 bp, synthetic construct
  source 1..32: mol_type = other DNA
agggatttagtagaagttgcaacactgaaagc

SEQ ID NO: 12 - DNA, 32 bp, synthetic construct
  source 1..32: mol_type = other DNA
tcctgagattctttgatacattttttctggcc

SEQ ID NO: 13 - DNA, 32 bp, synthetic construct
  source 1..32: mol_type = other DNA
accgagtatccatcactatttacacaccagtc

SEQ ID NO: 14 - DNA, 32 bp, synthetic construct
  source 1..32: mol_type = other DNA
cctcctcaccgggggtgtttctttggtatgag

SEQ ID NO: 15 - DNA, 32 bp, synthetic construct
  source 1..32: mol_type = other DNA
gctcgaatccagaatgtggtgtgtgctttcgc

SEQ ID NO: 16 - DNA, 32 bp, synthetic construct
  source 1..32: mol_type = other DNA
tcctgtgtctgcgcgcgatgccggggtgtcca

SEQ ID NO: 17 - DNA, 39 bp, synthetic construct
  source 1..39: mol_type = other DNA
cttgcctgtagacaggcgtataacgggaagaaagcgaaa

SEQ ID NO: 18 - DNA, 32 bp, synthetic construct
  source 1..32: mol_type = other DNA
agcaatacagtgttttagggcgcgcgctggca

SEQ ID NO: 19 - DNA, 32 bp, synthetic construct
  source 1..32: mol_type = other DNA
cggtcatacagttgagtcgggaaagcgtattg

SEQ ID NO: 20 - DNA, 31 bp, synthetic construct
  source 1..31: mol_type = other DNA
tgctgcggtcgtaatcaattgcgaccagtga

SEQ ID NO: 21 - DNA, 32 bp, synthetic construct
  source 1..32: mol_type = other DNA
cagtgtcagaaattgttggggtgctcaccgcc

SEQ ID NO: 22 - DNA, 32 bp, synthetic construct
  source 1..32: mol_type = other DNA
atcgtctggccgctactataatcagtgaggcc

SEQ ID NO: 23 - DNA, 32 bp, synthetic construct
  source 1..32: mol_type = other DNA
gtaagaattggtcagtagcatcaccttgctga

SEQ ID NO: 24 - DNA, 24 bp, synthetic construct
  source 1..24: mol_type = other DNA
ccgggtcagagagataaacgcggt

SEQ ID NO: 25 - DNA, 31 bp, synthetic construct
  source 1..31: mol_type = other DNA
cacgcaacagcagttgtacatcgacataaaa

SEQ ID NO: 26 - DNA, 32 bp, synthetic construct
  source 1..32: mol_type = other DNA
gtctttaaaaatctaatggcaaattattaaat

SEQ ID NO: 27 - DNA, 32 bp, synthetic construct
  source 1..32: mol_type = other DNA
catcgccaagtgccacaggttatctattagac

SEQ ID NO: 28 - DNA, 32 bp, synthetic construct
  source 1..32: mol_type = other DNA
gcagaagagtgaggcgaactaatagtcaatag

SEQ ID NO: 29 - DNA, 32 bp, synthetic construct
  source 1..32: mol_type = other DNA
cggccagattccggcagactttctaaacgtac

SEQ ID NO: 30 - DNA, 32 bp, synthetic construct
  source 1..32: mol_type = other DNA
cggacttgtgaagggtggaaaaagggaacgga

SEQ ID NO: 31 - DNA, 32 bp, synthetic construct
  source 1..32: mol_type = other DNA
ctggtcagtaaaaaaacttaaattgtgccaag

SEQ ID NO: 32 - DNA, 32 bp, synthetic construct
  source 1..32: mol_type = other DNA
caaatgaatgcgcgaacttctgacggaaaaac

SEQ ID NO: 33 - DNA, 32 bp, synthetic construct
  source 1..32: mol_type = other DNA
cctgcaacttaaaaataagggacagacgctca

SEQ ID NO: 34 - DNA, 32 bp, synthetic construct
  source 1..32: mol_type = other DNA
gattgccggcacatccgcggttgcgctcgtca

SEQ ID NO: 35 - DNA, 30 bp, synthetic construct
  source 1..30: mol_type = other DNA
tttagtgatagaacgttgcaggctcagcaa

SEQ ID NO: 36 - DNA, 32 bp, synthetic construct
  source 1..32: mol_type = other DNA
aaatcccgcagcaacccggctggagttacctg

SEQ ID NO: 37 - DNA, 32 bp, synthetic construct
  source 1..32: mol_type = other DNA
ctttaggaagtaataaaccgaacgaaccacca

SEQ ID NO: 38 - DNA, 24 bp, synthetic construct
  source 1..24: mol_type = other DNA
agcgccatcctgtagctggtgccg

SEQ ID NO: 39 - DNA, 32 bp, synthetic construct
  source 1..32: mol_type = other DNA
cacgacgtgtcacgttggcgcatcgtaaccgt

SEQ ID NO: 40 - DNA, 32 bp, synthetic construct
  source 1..32: mol_type = other DNA
tatcatttcaaaattagatgaataatcaagaa

SEQ ID NO: 41 - DNA, 32 bp, synthetic construct
  source 1..32: mol_type = other DNA
aggagcggtgaataatcgggagaatacctgag

SEQ ID NO: 42 - DNA, 32 bp, synthetic construct
  source 1..32: mol_type = other DNA
cagatgatcaatataatttgaataaaatcgcg

SEQ ID NO: 43 - DNA, 32 bp, synthetic construct
  source 1..32: mol_type = other DNA
ggctgcgcaccgcttccagctttcaataggaa

SEQ ID NO: 44 - DNA, 32 bp, synthetic construct
  source 1..32: mol_type = other DNA
cgggcctccaggaagaacaacccgaaattttt

SEQ ID NO: 45 - DNA, 32 bp, synthetic construct
  source 1..32: mol_type = other DNA
aagggggacagtttgaggcggatttaaacgtt

SEQ ID NO: 46 - DNA, 32 bp, synthetic construct
  source 1..32: mol_type = other DNA
taccatattgcggaacacaactcgcaacagtt

SEQ ID NO: 47 - DNA, 32 bp, synthetic construct
  source 1..32: mol_type = other DNA
tatacttcaattatcatttagaagtaaaatat

SEQ ID NO: 48 - DNA, 32 bp, synthetic construct
  source 1..32: mol_type = other DNA
tttccggcaactgttgaatcggcgccgtggtg

SEQ ID NO: 49 - DNA, 30 bp, synthetic construct
  source 1..30: mol_type = other DNA
atcggcctttcgctaccgccacgagacgca

SEQ ID NO: 50 - DNA, 32 bp, synthetic construct
  source 1..32: mol_type = other DNA
gcatctgctgtgctgcgacggccatctgctca

SEQ ID NO: 51 - DNA, 32 bp, synthetic construct
  source 1..32: mol_type = other DNA
ggattcgctttgaggatcatattcctgattat

SEQ ID NO: 52 - DNA, 32 bp, synthetic construct
  source 1..32: mol_type = other DNA
ctggccttgtttaccacgccattcgccattca

SEQ ID NO: 53 - DNA, 32 bp, synthetic construct
  source 1..32: mol_type = other DNA
tgggatagtgtaaaacaaggcgattaagttgg

SEQ ID NO: 54 - DNA, 24 bp, synthetic construct
  source 1..24: mol_type = other DNA
cgccatcataccaaaagagggtag

SEQ ID NO: 55 - DNA, 32 bp, synthetic construct
  source 1..32: mol_type = other DNA
ttgtataagcaatgccgtaggtaaagattcaa

SEQ ID NO: 56 - DNA, 32 bp, synthetic construct
  source 1..32: mol_type = other DNA
ttttaatgatttatcataactatataagaata

SEQ ID NO: 57 - DNA, 32 bp, synthetic construct
  source 1..32: mol_type = other DNA
tgtgagtgagattaagtcgcaagaataccgac

SEQ ID NO: 58 - DNA, 32 bp, synthetic construct
  source 1..32: mol_type = other DNA
cgctattaccttagaaaaatatatttcatctt

SEQ ID NO: 59 - DNA, 40 bp, synthetic construct
  source 1..40: mol_type = other DNA
ggctatcaggtcattgatgccggaacattatgaagcaata

SEQ ID NO: 60 - DNA, 32 bp, synthetic construct
  source 1..32: mol_type = other DNA
gaatcgattatgatatagcctttatcatacag

SEQ ID NO: 61 - DNA, 32 bp, synthetic construct
  source 1..32: mol_type = other DNA
tgtcaatcgaaaggccttagaaccactaatag

SEQ ID NO: 62 - DNA, 32 bp, synthetic construct
  source 1..32: mol_type = other DNA
aatagtgagaaacagtaaacaaactacagtaa

SEQ ID NO: 63 - DNA, 32 bp, synthetic construct
  source 1..32: mol_type = other DNA
gatagcttaataacctatttcaatacaataac

SEQ ID NO: 64 - DNA, 32 bp, synthetic construct
  source 1..32: mol_type = other DNA
ataaattacctgagagttttaaccatcaacat

SEQ ID NO: 65 - DNA, 30 bp, synthetic construct
  source 1..30: mol_type = other DNA
accatcaagaacggtttcgcatttcggatt

SEQ ID NO: 66 - DNA, 32 bp, synthetic construct
  source 1..32: mol_type = other DNA
aagggtgaatatgtacttaaattggaccgtaa

SEQ ID NO: 67 - DNA, 32 bp, synthetic construct
  source 1..32: mol_type = other DNA
gcgagaaaaattattctgcttctgtaaatcgt

SEQ ID NO: 68 - DNA, 24 bp, synthetic construct
  source 1..24: mol_type = other DNA
aagcctcaagcaaagctgttttaa

SEQ ID NO: 69 - DNA, 31 bp, synthetic construct
  source 1..31: mol_type = other DNA
gctgaaacaaactccgattagagagtacctt

SEQ ID NO: 70 - DNA, 32 bp, synthetic construct
  source 1..32: mol_type = other DNA
atatgcgtaaaaggtagcgcctgtcgagaaca

SEQ ID NO: 71 - DNA, 32 bp, synthetic construct
  source 1..32: mol_type = other DNA
agccaacgagccagtaaacaagaagaacgggt

SEQ ID NO: 72 - DNA, 40 bp, synthetic construct
  source 1..40: mol_type = other DNA
atcgccatgccaacatgagcatgtcaataatcggctgtct

SEQ ID NO: 73 - DNA, 48 bp, synthetic construct
  source 1..48: mol_type = other DNA
ctggaagtttcattccgctcaacaggattgcatcaaaaatcaggtctt

SEQ ID NO: 74 - DNA, 32 bp, synthetic construct
  source 1..32: mol_type = other DNA
gcgaacgacttagagcaaagactttaaacagt

SEQ ID NO: 75 - DNA, 32 bp, synthetic construct
  source 1..32: mol_type = other DNA
tacatttcccttttgacttcaaagtaaatatt

SEQ ID NO: 76 - DNA, 32 bp, synthetic construct
  source 1..32: mol_type = other DNA
gtaccgactatacaaagcgttaaatgtaaatg

SEQ ID NO: 77 - DNA, 32 bp, synthetic construct
  source 1..32: mol_type = other DNA
cattttcgctcaacagggtttgaacaaagaac

SEQ ID NO: 78 - DNA, 32 bp, synthetic construct
  source 1..32: mol_type = other DNA
atgctgtaatataacagcaaaattaccctgta

SEQ ID NO: 79 - DNA, 30 bp, synthetic construct
  source 1..30: mol_type = other DNA
gcggatgggtagattccaataaatttcaac

SEQ ID NO: 80 - DNA, 32 bp, synthetic construct
  source 1..32: mol_type = other DNA
taattgctgcaaatggtcaattctctcatata

SEQ ID NO: 81 - DNA, 32 bp, synthetic construct
  source 1..32: mol_type = other DNA
tcccatccaatttaattagggcttaattgaga

SEQ ID NO: 82 - DNA, 40 bp, synthetic construct
  source 1..40: mol_type = other DNA
ttccttataacgcgaggcgttttagcgaacctcccgactt

SEQ ID NO: 83 - DNA, 48 bp, synthetic construct
  source 1..48: mol_type = other DNA
taccctgactaccaatagaaattatagtcagagagcataatacggtgt

SEQ ID NO: 84 - DNA, 32 bp, synthetic construct
  source 1..32: mol_type = other DNA
gcgtccaatactgcggtgccagagggggtaat

SEQ ID NO: 85 - DNA, 32 bp, synthetic construct
  source 1..32: mol_type = other DNA
ccaatagcaagcaaatgcactcatttatcaac

SEQ ID NO: 86 - DNA, 32 bp, synthetic construct
  source 1..32: mol_type = other DNA
tatccggtattctaagcattccaaaaataata

SEQ ID NO: 87 - DNA, 48 bp, synthetic construct
  source 1..48: mol_type = other DNA
attacgaggcatagtaagagcaacactatcataccataaatcaaaaag

SEQ ID NO: 88 - DNA, 31 bp, synthetic construct
  source 1..31: mol_type = other DNA
acgacgataaaaaccaaaatgcttcaaatat

SEQ ID NO: 89 - DNA, 32 bp, synthetic construct
  source 1..32: mol_type = other DNA
tttgcaaaagaagtttaatcgtcacgaaccag

SEQ ID NO: 90 - DNA, 32 bp, synthetic construct
  source 1..32: mol_type = other DNA
tttaggaataccacattcaactaaatggttta

SEQ ID NO: 91 - DNA, 30 bp, synthetic construct
  source 1..30: mol_type = other DNA
tattacaggtagaaagattcatctacctta

SEQ ID NO: 92 - DNA, 32 bp, synthetic construct
  source 1..32: mol_type = other DNA
taaaacgaactaacggataccagtcaggacgt

SEQ ID NO: 93 - DNA, 24 bp, synthetic construct
  source 1..24: mol_type = other DNA
ctcgttaggccagccaaactcaaa

SEQ ID NO: 94 - DNA, 24 bp, synthetic construct
  source 1..24: mol_type = other DNA
accggaagaggtggcatcaataac

SEQ ID NO: 95 - DNA, 32 bp, synthetic construct
  source 1..32: mol_type = other DNA
cctttgcctaacgtcatttgcacgtaaaacag

SEQ ID NO: 96 - DNA, 40 bp, synthetic construct
  source 1..40: mol_type = other DNA
gataacccccatattatttatcccttaccaacgctaacga

SEQ ID NO: 97 - DNA, 31 bp, synthetic construct
  source 1..31: mol_type = other DNA
tcagaggcgattttttgtttaactttgcacc

SEQ ID NO: 98 - DNA, 32 bp, synthetic construct
  source 1..32: mol_type = other DNA
gctcattctttaatcattgtgaatagttgaga

SEQ ID NO: 99 - DNA, 32 bp, synthetic construct
  source 1..32: mol_type = other DNA
tattcatttaagaactggctcattaacaacat

SEQ ID NO: 100 - DNA, 31 bp, synthetic construct
  source 1..31: mol_type = other DNA
cgccagcatacatggcttttgattgccccct

SEQ ID NO: 101 - DNA, 40 bp, synthetic construct
  source 1..40: mol_type = other DNA
agacgattagtctctgaatttacctgaaacatgaaagtat

SEQ ID NO: 102 - DNA, 23 bp, synthetic construct
  source 1..23: mol_type = other DNA
ggagcgggaaagggcgaaaaacc

SEQ ID NO: 103 - DNA, 32 bp, synthetic construct
  source 1..32: mol_type = other DNA
agtgtagcggtcacgcgtccactattaaagaa

SEQ ID NO: 104 - DNA, 32 bp, synthetic construct
  source 1..32: mol_type = other DNA
gcaaggcagaagcccgttaattgctgaatata

SEQ ID NO: 105 - DNA, 31 bp, synthetic construct
  source 1..31: mol_type = other DNA
tagtagcaaattcgagtaagaggtcattttt

SEQ ID NO: 106 - DNA, 32 bp, synthetic construct
  source 1..32: mol_type = other DNA
agcaagccgtttttatggaatcattaccgcgc

SEQ ID NO: 107 - DNA, 30 bp, synthetic construct
  source 1..30: mol_type = other DNA
attaaaccaagtacccagatatagaaggct

SEQ ID NO: 108 - DNA, 32 bp, synthetic construct
  source 1..32: mol_type = other DNA
tcagaaaacgagaatgaaccctcgtttaccag

SEQ ID NO: 109 - DNA, 30 bp, synthetic construct
  source 1..30: mol_type = other DNA
cattgaatccccctcaaatagcgagaggct

SEQ ID NO: 110 - DNA, 24 bp, synthetic construct
  source 1..24: mol_type = other DNA
aacaaaatgggttataaaatcata

SEQ ID NO: 111 - DNA, 24 bp, synthetic construct
  source 1..24: mol_type = other DNA
ccggcgaacgtggcgactaaaggg

SEQ ID NO: 112 - DNA, 24 bp, synthetic construct
  source 1..24: mol_type = other DNA
cagccagcgtaaagcctatccgct

SEQ ID NO: 113 - DNA, 24 bp, synthetic construct
  source 1..24: mol_type = other DNA
tttgccgcccagcttagcaagaat

SEQ ID NO: 114 - DNA, 24 bp, synthetic construct
  source 1..24: mol_type = other DNA
ttttaaatgcaaatatcccggttg

SEQ ID NO: 115 - DNA, 24 bp, synthetic construct
  source 1..24: mol_type = other DNA
aacaccggtgcagaacaagtaatt

SEQ ID NO: 116 - DNA, 24 bp, synthetic construct
  source 1..24: mol_type = other DNA
cttgacaatgtacagaccaggcgc

SEQ ID NO: 117 - DNA, 24 bp, synthetic construct
  source 1..24: mol_type = other DNA
tgacccccaacctaaaacgaaaga

SEQ ID NO: 118 - DNA, 32 bp, synthetic construct
  source 1..32: mol_type = other DNA
atattcggtcgctgagccgacaatgacaacaa

SEQ ID NO: 119 - DNA, 24 bp, synthetic construct
  source 1..24: mol_type = other DNA
ttcaacagagacgttagtaaatga

SEQ ID NO: 120 - DNA, 24 bp, synthetic construct
  source 1..24: mol_type = other DNA
accctcagtatcaccgtactcagg

SEQ ID NO: 121 - DNA, 32 bp, synthetic construct
  source 1..32: mol_type = other DNA
cggggagaagggttgagtgttgttaaggatta

SEQ ID NO: 122 - DNA, 32 bp, synthetic construct
  source 1..32: mol_type = other DNA
aaagatgtaatcacacaccaccggccaacgcg

SEQ ID NO: 123 - DNA, 24 bp, synthetic construct
  source 1..24: mol_type = other DNA
gcacgcgtaatcaccattcgtcct

SEQ ID NO: 124 - DNA, 32 bp, synthetic construct
  source 1..32: mol_type = other DNA
ctggtaatcattaatgtcttcgcgtccgtgag

SEQ ID NO: 125 - DNA, 24 bp, synthetic construct
  source 1..24: mol_type = other DNA
taaaatctctgagattttggccgg

SEQ ID NO: 126 - DNA, 24 bp, synthetic construct
  source 1..24: mol_type = other DNA
ccgttttttcactccaaaaggtag

SEQ ID NO: 127 - DNA, 40 bp, synthetic construct
  source 1..40: mol_type = other DNA
gattaccggaatttgtctgttgcccgtcgctggcagcctc

SEQ ID NO: 128 - DNA, 24 bp, synthetic construct
  source 1..24: mol_type = other DNA
gaaaccaggtaacagacggctaat

SEQ ID NO: 129 - DNA, 24 bp, synthetic construct
  source 1..24: mol_type = other DNA
ctatttttcgccatgttgctcaat

SEQ ID NO: 130 - DNA, 40 bp, synthetic construct
  source 1..40: mol_type = other DNA
tttagtaaatcggttgaaaataattcgttacaccaagcgt

SEQ ID NO: 131 - DNA, 24 bp, synthetic construct
  source 1..24: mol_type = other DNA
atatgcaataagagtaagaacaaa

SEQ ID NO: 132 - DNA, 48 bp, synthetic construct
  source 1..48: mol_type = other DNA
caaaaggagcgggagggaataacactaacaacatttaaagagcttaat

SEQ ID NO: 133 - DNA, 40 bp, synthetic construct
  source 1..40: mol_type = other DNA
cagggaagcgaggaaagagttttcattaaagatctacaaa

SEQ ID NO: 134 - DNA, 40 bp, synthetic construct
  source 1..40: mol_type = other DNA
aataacgggagggaaggcattcatggcaaaaggtcgagcc

SEQ ID NO: 135 - DNA, 24 bp, synthetic construct
  source 1..24: mol_type = other DNA
attgacggattttcggtcgcagag

SEQ ID NO: 136 - DNA, 24 bp, synthetic construct
  source 1..24: mol_type = other DNA
cccccttaaacaaatagccgtctg

SEQ ID NO: 137 - DNA, 24 bp, synthetic construct
  source 1..24: mol_type = other DNA
cattaaagctcaagagccagtttg

SEQ ID NO: 138 - DNA, 24 bp, synthetic construct
  source 1..24: mol_type = other DNA
tacagagattttgaagccttaaat

SEQ ID NO: 139 - DNA, 31 bp, synthetic construct
  source 1..31: mol_type = other DNA
acaacgctgaaaatctccaaaaaaaaggagc

SEQ ID NO: 140 - DNA, 40 bp, synthetic construct
  source 1..40: mol_type = other DNA
taagaggctgagactcccagaatggaaagcgcggccttga

SEQ ID NO: 141 - DNA, 41 bp, synthetic construct
  source 1..41: mol_type = other DNA
ggattagcggggtttttaccgtaacactgagtgtacaaact

SEQ ID NO: 142 - DNA, 24 bp, synthetic construct
  source 1..24: mol_type = other DNA
ggcttgagtgcagatacataacgc

SEQ ID NO: 143 - DNA, 32 bp, synthetic construct
  source 1..32: mol_type = other DNA
aaggaaaccgcattagacgggagagcagcctt

SEQ ID NO: 144 - DNA, 32 bp, synthetic construct
  source 1..32: mol_type = other DNA
cggaacgacctgacgagaaacaccgtaaattg

SEQ ID NO: 145 - DNA, 32 bp, synthetic construct
  source 1..32: mol_type = other DNA
gattgaggaatacccaaaagaactgttaccag

SEQ ID NO: 146 - DNA, 32 bp, synthetic construct
  source 1..32: mol_type = other DNA
ggactaaagtcgaaatccgcgacctacttagc

SEQ ID NO: 147 - DNA, 32 bp, synthetic construct
  source 1..32: mol_type = other DNA
tcatcggcaaattattcattaaagattcaacc

SEQ ID NO: 148 - DNA, 32 bp, synthetic construct
  source 1..32: mol_type = other DNA
ctttaattggaacgagggtagcaaggctttga

SEQ ID NO: 149 - DNA, 32 bp, synthetic construct
  source 1..32: mol_type = other DNA
tattcacattagcgtttgccatctgcgcgttt

SEQ ID NO: 150 - DNA, 24 bp, synthetic construct
  source 1..24: mol_type = other DNA
accggaagaggtggcatcaataac

SEQ ID NO: 151 - DNA, 24 bp, synthetic construct
  source 1..24: mol_type = other DNA
ctcgttaggccagccaaactcaaa

SEQ ID NO: 152 - DNA, 32 bp, synthetic construct; identical to SEQ ID NO: 95
  source 1..32: mol_type = other DNA

SEQ ID NO: 153 - DNA, 30 bp, synthetic construct
  source 1..30: mol_type = other DNA
aatagataaaataagttcttaccagtataa

SEQ ID NO: 154 - DNA, 31 bp, synthetic construct
  source 1..31: mol_type = other DNA
tgagctaacggcatcactgtgcactctgtgg

SEQ ID NO: 155 - DNA, 31 bp, synthetic construct
  source 1..31: mol_type = other DNA
ctttcagagaacaaacggggacgacgacagt

SEQ ID NO: 156 - DNA, 15 bp, synthetic construct
  source 1..15: mol_type = other DNA
cccgacggggaaagc

SEQ ID NO: 157 - DNA, 15 bp, synthetic construct
  source 1..15: mol_type = other DNA
cccccgagccggaag

SEQ ID NO: 158 - DNA, 15 bp, synthetic construct
  source 1..15: mol_type = other DNA
ccctatccagaacaa

SEQ ID NO: 159 - DNA, 15 bp, synthetic construct
  source 1..15: mol_type = other DNA
cccgtggtgccatcc

SEQ ID NO: 160 - DNA, 15 bp, synthetic construct
  source 1..15: mol_type = other DNA
cccccaaaccctcaa

SEQ ID NO: 161 - DNA, 15 bp, synthetic construct
  source 1..15: mol_type = other DNA
ccccgttttcccagt

SEQ ID NO: 162 - DNA, 15 bp, synthetic construct
  source 1..15: mol_type = other DNA
gtaacgccaggcccc

SEQ ID NO: 163 - DNA, 15 bp, synthetic construct
  source 1..15: mol_type = other DNA
aaataaagaaacccc

SEQ ID NO: 164 - DNA, 15 bp, synthetic construct
  source 1..15: mol_type = other DNA
ccccttgcgtagatt

SEQ ID NO: 165 - DNA, 15 bp, synthetic construct
  source 1..15: mol_type = other DNA
ccccaaacaggaaga

SEQ ID NO: 166 - DNA, 15 bp, synthetic construct
  source 1..15: mol_type = other DNA
cccttaacctccggc

SEQ ID NO: 167 - DNA, 15 bp, synthetic construct
  source 1..15: mol_type = other DNA
ccctttggggcgcga

SEQ ID NO: 168 - DNA, 15 bp, synthetic construct
  source 1..15: mol_type = other DNA
cccaaacaacatgtt

SEQ ID NO: 169 - DNA, 15 bp, synthetic construct
  source 1..15: mol_type = other DNA
cccctagactggata

SEQ ID NO: 170 - DNA, 15 bp, synthetic construct
  source 1..15: mol_type = other DNA
agtaaaatgttcccc

SEQ ID NO: 171 - DNA, 24 bp, synthetic construct
  source 1..24: mol_type = other DNA
gcgtctttccagagcctaattccc

SEQ ID NO: 172 - DNA, 15 bp, synthetic construct
  source 1..15: mol_type = other DNA
ccccatctacgttaa

SEQ ID NO: 173 - DNA, 15 bp, synthetic construct
  source 1..15: mol_type = other DNA
tgggaagaaaacccc

SEQ ID NO: 174 - DNA, 16 bp, synthetic construct
  source 1..16: mol_type = other DNA
tgagttaagcccaccc

SEQ ID NO: 175 - DNA, 15 bp, synthetic construct
  source 1..15: mol_type = other DNA
ataggctggctcccc

SEQ ID NO: 176 - DNA, 16 bp, synthetic construct
  source 1..16: mol_type = other DNA
tataaaagaaacgccc

SEQ ID NO: 177 - DNA, 48 bp, synthetic construct
  source 1..48: mol_type = other DNA
ccccaaagacaccacggaataagtcaccattaccattagcaaggcccc

SEQ ID NO: 178 - DNA, 15 bp, synthetic construct
  source 1..15: mol_type = other DNA
ggcaaaagaatcccc

SEQ ID NO: 179 - DNA, 15 bp, synthetic construct
  source 1..15: mol_type = other DNA
ccccgcataaccgat

SEQ ID NO: 180 - DNA, 48 bp, synthetic construct
  source 1..48: mol_type = other DNA
ccccggaaacgtcaccaatgaaaccctcagaaccgccaccctcagccc

SEQ ID NO: 181 - DNA, 15 bp, synthetic construct
  source 1..15: mol_type = other DNA
ccatcgcccaccccc

SEQ ID NO: 182 - DNA, 15 bp, synthetic construct
  source 1..15: mol_type = other DNA
attttctgtatcccc

SEQ ID NO: 183 - DNA, 15 bp, synthetic construct
  source 1..15: mol_type = other DNA
aggtttagtaccccc

SEQ ID NO: 184 - DNA, 32 bp, synthetic construct
  source 1..32: mol_type = other DNA
cataaagggaaatagcaatagctaatcagaga

SEQ ID NO: 185 - DNA, 32 bp, synthetic construct
  source 1..32: mol_type = other DNA
accagtagttattttgtcacaatcaatacata

SEQ ID NO: 186 - DNA, 32 bp, synthetic construct
  source 1..32: mol_type = other DNA
gccgccaccatcgatagcagcaccgcaaaatc

SEQ ID NO: 187 - DNA, 32 bp, synthetic construct
  source 1..32: mol_type = other DNA
agtgtactcaccagaaccaccaccccctcaga

SEQ ID NO: 188 - DNA, 24 bp, synthetic construct
  source 1..24: mol_type = other DNA
ccgtataaacagttaagatacagg

SEQ ID NO: 189 - DNA, 31 bp, synthetic construct
  source 1..31: mol_type = other DNA
cagctacaattttatcctgaatcaatccaaa

SEQ ID NO: 190 - DNA, 31 bp, synthetic construct
  source 1..31: mol_type = other DNA
taagaaagtaattgagcgctaattcttaccg

SEQ ID NO: 191 - DNA, 31 bp, synthetic construct
  source 1..31: mol_type = other DNA
aagcccttttagcaaacgtagaaaatagaaa

SEQ ID NO: 192 - DNA, 31 bp, synthetic construct
  source 1..31: mol_type = other DNA
attcatattgggaattagagccagtaatcag

SEQ ID NO: 193 - DNA, 31 bp, synthetic construct
  source 1..31: mol_type = other DNA
tagcgacaccaccggaaccgcctagagccgc

SEQ ID NO: 194 - DNA, 31 bp, synthetic construct
  source 1..31: mol_type = other DNA
gcagtatgtttaagaaaagtaaggaacaaag

SEQ ID NO: 195 - DNA, 31 bp, synthetic construct
  source 1..31: mol_type = other DNA
gagccattggtttaccagcgccacttattac

SEQ ID NO: 196 - DNA, 31 bp, synthetic construct
  source 1..31: mol_type = other DNA
cagagccagaatcaagtttgcctaccgactt

SEQ ID NO: 197 - DNA, 31 bp, synthetic construct
  source 1..31: mol_type = other DNA
aagcgtcattgacaggaggttgaaccggaac

SEQ ID NO: 198 - DNA, 31 bp, synthetic construct
  source 1..31: mol_type = other DNA
gcctatttcggaacctattattcgttccagt

SEQ ID NO: 199 - DNA, 24 bp, synthetic construct
  source 1..24: mol_type = other DNA
caagattagttgctatgtcaaaaa

SEQ ID NO: 200 - DNA, 32 bp, synthetic construct
  source 1..32: mol_type = other DNA
tgaaaataattaactgaacaccctcagatagc

SEQ ID NO: 201 - DNA, 32 bp, synthetic construct
  source 1..32: mol_type = other DNA
cgaacaaaggcatgattaagactcaagacaaa

SEQ ID NO: 202 - DNA, 32 bp, synthetic construct
  source 1..32: mol_type = other DNA
agggcgacgtgaattatcaccgtcttagcgtc

SEQ ID NO: 203 - DNA, 32 bp, synthetic construct
  source 1..32: mol_type = other DNA
agactgtatttcataatcaaaatcggcaggtc

SEQ ID NO: 204 - DNA, 32 bp, synthetic construct
  source 1..32: mol_type = other DNA
atttcaacagtgaataaggcttgcggcgcaga

SEQ ID NO: 205 - DNA, 32 bp, synthetic construct
  source 1..32: mol_type = other DNA
cggtcaattcgcctgataaattgtgacttttt

SEQ ID NO: 206 - DNA, 32 bp, synthetic construct
  source 1..32: mol_type = other DNA
catgaggaagcgaaagacagcatcgtatcggt

SEQ ID NO: 207 - DNA, 32 bp, synthetic construct
  source 1..32: mol_type = other DNA
ttatcagcaataattttttcacgtctgtagca

SEQ ID NO: 208 - DNA, 32 bp, synthetic construct
  source 1..32: mol_type = other DNA
ttccacagccaataggaacccatggctcagta

SEQ ID NO: 209 - DNA, 32 bp, synthetic construct
  source 1..32: mol_type = other DNA
ttgtatcacataagggaaccgaacacaaagct

SEQ ID NO: 210 - DNA, 32 bp, synthetic construct
  source 1..32: mol_type = other DNA
ccctcagcagtttccattaaacggacggagat

SEQ ID NO: 211 - DNA, 32 bp, synthetic construct
  source 1..32: mol_type = other DNA
ttgcgaatttgctttcgaggtgaagatcgtca

SEQ ID NO: 212 - DNA, 32 bp, synthetic construct
  source 1..32: mol_type = other DNA
tagcaagcacagccctcatagttataaaggaa

SEQ ID NO: 213 - DNA, 32 bp, synthetic construct
  source 1..32: mol_type = other DNA
ccaggcggataagtgccgtcgagattcaggga

SEQ ID NO: 214 - DNA, 30 bp, synthetic construct
  source 1..30: mol_type = other DNA
tgcgatttacccaaatcaacgtatgaccaa

SEQ ID NO: 215 - DNA, 30 bp, synthetic construct
  source 1..30: mol_type = other DNA
ctttgaaagcgaaacaaagtacagtaaaat

SEQ ID NO: 216 - DNA, 30 bp, synthetic construct
  source 1..30: mol_type = other DNA
acgtaatgaggccgcttttgcggtttctta

SEQ ID NO: 217 - DNA, 30 bp, synthetic construct
  source 1..30: mol_type = other DNA
aacagcttatagaaaggaacaacgcgtaac

SEQ ID NO: 218 - DNA, 30 bp, synthetic construct
  source 1..30: mol_type = other DNA
gatctaaagccaccaccctcattgggttga

SEQ ID NO: 219 - DNA, 32 bp, synthetic construct
  source 1..32: mol_type = other DNA
taccaagcgaggacagatgaacgggaaccgga

SEQ ID NO: 220 - DNA, 32 bp, synthetic construct
  source 1..32: mol_type = other DNA
ggagttaaccactacgaaggcaccagcgatta

SEQ ID NO: 221 - DNA, 32 bp, synthetic construct
  source 1..32: mol_type = other DNA
gagtgagagataccgatagttgcggcttgcag

SEQ ID NO: 222 - DNA, 32 bp, synthetic construct
  source 1..32: mol_type = other DNA
ccctcagagttttgtcgtctttcctttcagcg

SEQ ID NO: 223 - DNA, 32 bp, synthetic construct
  source 1..32: mol_type = other DNA
tataagtatagcccggaataggtgaaccgcca

SEQ ID NO: 224 - DNA, 32 bp, synthetic construct
  source 1..32: mol_type = other DNA
atattaccaatcagagacaggaggccgattaa

SEQ ID NO: 225 - DNA, 32 bp, synthetic construct
  source 1..32: mol_type = other DNA
ttcaggttcgaacgttaaagtttgagtaacat

SEQ ID NO: 226 - DNA, 32 bp, synthetic construct
  source 1..32: mol_type = other DNA
cttaggtttaattacatcatttgaattacctt

SEQ ID NO: 227 - DNA, 32 bp, synthetic construct
  source 1..32: mol_type = other DNA
tcaatatcacgtggcattttgaatggctatta

SEQ ID NO: 228 - DNA, 32 bp, synthetic construct
  source 1..32: mol_type = other DNA
tcagctaaaatcataaaagcctgtttagtatc

SEQ ID NO: 229 - DNA, 30 bp, synthetic construct
  source 1..30: mol_type = other DNA
ttgctttgaaataccttagtaataacatca

SEQ ID NO: 230 - DNA, 30 bp, synthetic construct
  source 1..30: mol_type = other DNA
aacagagattgaggagctgagagccagcag

SEQ ID NO: 231 - DNA, 30 bp, synthetic construct
  source 1..30: mol_type = other DNA
tttacaaatttacatggaagggttagaacc

SEQ ID NO: 232 - DNA, 30 bp, synthetic construct
  source 1..30: mol_type = other DNA
caaaagaaaatccaaacgctgagaagagtc

SEQ ID NO: 233 - DNA, 30 bp, synthetic construct
  source 1..30: mol_type = other DNA
cgtgtgatagtcctgataagagaatataaa

SEQ ID NO: 234 - DNA, 30 bp, synthetic construct
  source 1..30: mol_type = other DNA
gctcatggacgagcaaacggtacgccagaa

SEQ ID NO: 235 - DNA, 30 bp, synthetic construct
  source 1..30: mol_type = other DNA
gaaaggaatagaaccctgatagccctaaaa

SEQ ID NO: 236 - DNA, 30 bp, synthetic construct
  source 1..30: mol_type = other DNA
cagtacctcaattcgaaagaaaccaccaga

SEQ ID NO: 237 - DNA, 30 bp, synthetic construct
  source 1..30: mol_type = other DNA
ctgatgcagatgatgacataaatcaatata

SEQ ID NO: 238 - DNA, 30 bp, synthetic construct; identical to SEQ ID NO: 153
  source 1..30: mol_type = other DNA

SEQ ID NO: 239 - DNA, 32 bp, synthetic construct
  source 1..32: mol_type = other DNA
cttaatgcaaatggatgcaaattaaccgttgt

SEQ ID NO: 240 - DNA, 32 bp, synthetic construct
  source 1..32: mol_type = other DNA
acacgaccgcactaacgtcagtattaacaccg

SEQ ID NO: 241 - DNA, 32 bp, synthetic construct
  source 1..32: mol_type = other DNA
ataatacactgattgctcctgattgtttggat

SEQ ID NO: 242 - DNA, 32 bp, synthetic construct
  source 1..32: mol_type = other DNA
cagaggcgactttttctccttgaaaacatagc

SEQ ID NO: 243 - DNA, 32 bp, synthetic construct
  source 1..32: mol_type = other DNA
ctgacctataatttacgtaatttaggcagagg

SEQ ID NO: 244 - DNA, 32 bp, synthetic construct
  source 1..32: mol_type = other DNA
ggcgccagggtggtttatcccttataaatcaa

SEQ ID NO: 245 - DNA, 32 bp, synthetic construct
  source 1..32: mol_type = other DNA
actgcccgccttacaccggcgggccgttttca

SEQ ID NO: 246 - DNA, 32 bp, synthetic construct
  source 1..32: mol_type = other DNA
actcaatcgctctcacaaagttaaacgatgct

SEQ ID NO: 247 - DNA, 32 bp, synthetic construct
  source 1..32: mol_type = other DNA
taacctcaagcgagtatcgcactccagccagc

SEQ ID NO: 248 - DNA, 32 bp, synthetic construct
  source 1..32: mol_type = other DNA
gttaaatcgcgggagatcaaccgttctagctg

SEQ ID NO: 249 - DNA, 32 bp, synthetic construct
  source 1..32: mol_type = other DNA
taaacatcctttccaggatccccgggtaccga

SEQ ID NO: 250 - DNA, 32 bp, synthetic construct
  source 1..32: mol_type = other DNA
aagggatacgccgggctcataacggaacgtgc

SEQ ID NO: 251 - DNA, 32 bp, synthetic construct
  source 1..32: mol_type = other DNA
taaatgtgccggaaacggaagggcgatcggtg

SEQ ID NO: 252 - DNA, 32 bp, synthetic construct
  source 1..32: mol_type = other DNA
atacttttagctcatttctggagcaaacaaga

SEQ ID NO: 253 - DNA, 32 bp, synthetic construct
  source 1..32: mol_type = other DNA
attaagagaagaattagttgattcccaattct

SEQ ID NO: 254 - DNA, 31 bp, synthetic construct
  source 1..31: mol_type = other DNA
gacgggcaacagctgcctgtttgatggtggt

SEQ ID NO: 255 - DNA, 31 bp, synthetic construct; identical to SEQ ID NO: 154
  source 1..31: mol_type = other DNA

SEQ ID NO: 256 - DNA, 31 bp, synthetic construct
  source 1..31: mol_type = other DNA
gcatcagcggatcaaagccgcacaggcggcc

SEQ ID NO: 257 - DNA, 31 bp, synthetic construct; identical to SEQ ID NO: 155
  source 1..31: mol_type = other DNA

SEQ ID NO: 258 - DNA, 31 bp, synthetic construct
  source 1..31: mol_type = other DNA
aatattttaaaaatttggagacagtcaaatc

SEQ ID NO: 259 - DNA, 31 bp, synthetic construct
  source 1..31: mol_type = other DNA
atcgttaactcacattatggtcatagctgtt

SEQ ID NO: 260 - DNA, 31 bp, synthetic construct
  source 1..31: mol_type = other DNA
gaaacagcggggtcatcagcgtggtgctggt

SEQ ID NO: 261 - DNA, 31 bp, synthetic construct
  source 1..31: mol_type = other DNA
ctccgtggggtggagttacgccagctggcga

SEQ ID NO: 262 - DNA, 31 bp, synthetic construct
  source 1..31: mol_type = other DNA
gcaaggatgttaaaaaatcgtaaaactagca

SEQ ID NO: 263 - DNA, 31 bp, synthetic construct
  source 1..31: mol_type = other DNA
cgcgttttttaacattagtttgaccattaga

SEQ ID NO: 264 - DNA, 43 bp, synthetic construct
  source 1..43: mol_type = other DNA
agcccccgatttagagcttttgatcacttttgtgactatgcaa

SEQ ID NO: 265 - DNA, 43 bp, synthetic construct
  source 1..43: mol_type = other DNA
ctatcggccttgctggtaattgatcacttttgtgactatgcaa

SEQ ID NO: 266 - DNA, 43 bp, synthetic construct
  source 1..43: mol_type = other DNA
ggtctgagagactacctttttgatcacttttgtgactatgcaa

SEQ ID NO: 267 - DNA, 43 bp, synthetic construct
  source 1..43: mol_type = other DNA
ctgtccagacgacgacaatttgatcacttttgtgactatgcaa

SEQ ID NO: 268 - DNA, 45 bp, synthetic construct
  source 1..45: mol_type = other DNA
agtcacaaaagtgatctgccagttacaaaataaacagacaagaat

SEQ ID NO: 269 - DNA, 45 bp, synthetic construct
  source 1..45: mol_type = other DNA
agtcacaaaagtgatcataataagagcaagaaacaattggcaaca

SEQ ID NO: 270 - DNA, 53 bp, synthetic construct
  source 1..53: mol_type = other DNA
agtcacaaaagtgatcagccaccaccctcagagccgcggtaataagttttaac

SEQ ID NO: 271 - DNA, 37 bp, synthetic construct
  source 1..37: mol_type = other DNA
agtcacaaaagtgatccagtgccttgagtaacagtgc

SEQ ID NO: 272 - DNA, 42 bp, synthetic construct
  source 1..42: mol_type = other DNA
cacaattccacacaacataacgggtgcgatttctgtgtgaga

SEQ ID NO: 273 - DNA, 42 bp, synthetic construct
  source 1..42: mol_type = other DNA
gccaacggcagcaccgtcgacgggtgcgatttctgtgtgaga

SEQ ID NO: 274 - DNA, 42 bp, synthetic construct
  source 1..42: mol_type = other DNA
ataatcagaaaagccccaaacgggtgcgatttctgtgtgaga

SEQ ID NO: 275 - DNA, 42 bp, synthetic construct
  source 1..42: mol_type = other DNA
ctgtttagctatattttcaacgggtgcgatttctgtgtgaga

SEQ ID NO: 276 - DNA, 44 bp, synthetic construct
  source 1..44: mol_type = other DNA
acagaaatcgcacccgtttttttttgaccttcatcaagagtaat

SEQ ID NO: 277 - DNA, 43 bp, synthetic construct
  source 1..43: mol_type = other DNA
acagaaatcgcacccgttttttttacactaaaacactcatctt

SEQ ID NO: 278 - DNA, 43 bp, synthetic construct
  source 1..43: mol_type = other DNA
acagaaatcgcacccgttttttttgggattttgctaaacaact

SEQ ID NO: 279 - DNA, 43 bp, synthetic construct
  source 1..43: mol_type = other DNA
acagaaatcgcacccgttttttttcgccaccctcagaaccgcc

SEQ ID NO: 280 - DNA, 43 bp, synthetic construct
  source 1..43: mol_type = other DNA
agcccccgatttagagctttttcaacatcagtctgataagcta

SEQ ID NO: 281 - DNA, 43 bp, synthetic construct
  source 1..43: mol_type = other DNA
ctatcggccttgctggtaatttcaacatcagtctgataagcta

SEQ ID NO: 282 - DNA, 43 bp, synthetic construct
  source 1..43: mol_type = other DNA
ggtctgagagactaccttttttcaacatcagtctgataagcta

SEQ ID NO: 283 - DNA, 43 bp, synthetic construct
  source 1..43: mol_type = other DNA
ctgtccagacgacgacaattttcaacatcagtctgataagcta

SEQ ID NO: 284 - DNA, 53 bp, synthetic construct
  source 1..53: mol_type = other DNA
atcagactgatgttgatgccagttacaaaataaacagacaagaattgagttaa

SEQ ID NO: 285 - DNA, 45 bp, synthetic construct
  source 1..45: mol_type = other DNA
atcagactgatgttgaataataagagcaagaaacaattggcaaca

SEQ ID NO: 286 - DNA, 53 bp, synthetic construct
  source 1..53: mol_type = other DNA
atcagactgatgttgaagccaccaccctcagagccgcggtaataagttttaac

SEQ ID NO: 287 - DNA, 37 bp, synthetic construct
  source 1..37: mol_type = other DNA
atcagactgatgttgacagtgccttgagtaacagtgc

SEQ ID NO: 288 - DNA, 41 bp, synthetic construct
  source 1..41: mol_type = other DNA
cacaattccacacaacataaactatacaacctactacctca

SEQ ID NO: 289 - DNA, 41 bp, synthetic construct
  source 1..41: mol_type = other DNA
gccaacggcagcaccgtcgaactatacaacctactacctca

SEQ ID NO: 290 - DNA, 41 bp, synthetic construct
  source 1..41: mol_type = other DNA
ataatcagaaaagccccaaaactatacaacctactacctca

SEQ ID NO: 291 - DNA, 41 bp, synthetic construct
  source 1..41: mol_type = other DNA
ctgtttagctatattttcaaactatacaacctactacctca

SEQ ID NO: 292 - DNA, 43 bp, synthetic construct
  source 1..43: mol_type = other DNA
agtaggttgtatagttttttttttgaccttcatcaagagtaat

SEQ ID NO: 293 - DNA, 42 bp, synthetic construct
  source 1..42: mol_type = other DNA
agtaggttgtatagtttttttttacactaaaacactcatctt

SEQ ID NO: 294 - DNA, 42 bp, synthetic construct
  source 1..42: mol_type = other DNA
agtaggttgtatagtttttttttgggattttgctaaacaact

SEQ ID NO: 295 - DNA, 42 bp, synthetic construct
  source 1..42: mol_type = other DNA
agtaggttgtatagtttttttttcgccaccctcagaaccgcc

SEQ ID NO: 296 - DNA, 23 bp, synthetic construct
  source 1..23: mol_type = other DNA
tctcacacagaaatcgcacccgt

SEQ ID NO: 297 - DNA, 22 bp, synthetic construct
  source 1..22: mol_type = other DNA
ttgcatagtcacaaaagtgatc

SEQ ID NO: 298 - RNA, 22 nt, synthetic construct
  source 1..22: mol_type = other RNA
tgaggtagtaggttgtatagtt

SEQ ID NO: 299 - RNA, 22 nt, synthetic construct
  source 1..22: mol_type = other RNA
tcaacatcagtctgataagcta

SEQ ID NO: 300 - DNA, 21 bp, synthetic construct
  source 1..21: mol_type = other DNA
catcataattttaaaacaatt